European Patent Application EP 4 733 323 A1, published April 29, 2026. Title: 一种抗体或其抗原结合片段及其应用. Applicant: 森妙生物科技（西安）有限公司. The sequence listing filed with the application follows.

SEQUENCE LISTING (19 sequences)

SEQ ID NO: 1 - protein, 8 aa, synthetic construct
  SITE 2: note = I, S, F, T or V
  SITE 3: note = I, T or A
  SITE 6: note = G, N, S, V, L, A, D, Y or I
GXXFSXAW

SEQ ID NO: 2 - protein, 8 aa, synthetic construct
GTIFSDSF

SEQ ID NO: 3 - protein, 8 aa, synthetic construct
  SITE 4: note = G, A, S, D or T
  SITE 6: note = S, D, I, T, V or M
ITSXGXTV

SEQ ID NO: 4 - protein, 8 aa, synthetic construct
ITSGDITN

SEQ ID NO: 5 - protein, 10 aa, synthetic construct
NARPGAVNSY

SEQ ID NO: 6 - protein, 9 aa, synthetic construct
NSRIYTRSY

SEQ ID NO: 7 - protein, 12 aa, synthetic construct
NARPRGLSFSSY

SEQ ID NO: 8 - protein, 115 aa, synthetic construct
QLRLLESGGGLVQAGESLRLSCAVSGTIFSDSFLGWYRQAPGKQRELIASITSGGSTVYAGSVKGRFTISRDNAQDTVYLQMNSLKPEDTAVYYCNSRIYTRSYWGQGTQVTVSS

SEQ ID NO: 9 - protein, 118 aa, synthetic construct
QVQLVESGGGLVQAGGSLRLSCAASGIIFSGAWMGWYRQAAGEQRELVASITSGDITNYADSVKGRFTISRDNAENTGYLQMNTLKPEDTAVYYCNARPRGLSFSSYWGQGTLVTVSS

SEQ ID NO: 10 - DNA, 348 bp, synthetic construct
  source 1..348: mol_type = other DNA
caggtacagctgaaagagtctgggggaggcttggtgcaggctggggggtctctgagactctcctgtgtagcctctggattcacattcagtagcgcgtggatgggctggtaccgccaggctgcagggaagcagcgcgaattgttcgcatctattactagtagtggtgacacagtctatgcaggctccgtgaagggccgattctccatctctaagaacaacgccgagaacactctttatctgcaaatggatgcgctgaggcctgaagatacagccgtctattactgcaatgcccgtccgggggcggtcaatagttactggggccaggggacccaggtcaccgtctccaca

SEQ ID NO: 11 - DNA, 345 bp, synthetic construct
  source 1..345: mol_type = other DNA
cagttgcggctcttggagtctgggggaggcctggtgcaggctggggagtctctgagactctcctgtgctgtctctggaaccatctttagtgacagtttcctgggctggtaccgccaggctccagggaagcagcgcgagttgatcgcaagtattactagtggtggtagcacagtttatgcagggtccgtaaagggccgattcaccatctccagagacaacgcccaggacacggtgtatctgcaaatgaacagcctgaaacctgaggacacagccgtctattactgtaattcacgcatctatactcgatcctactggggccaggggacccaagtcaccgtctcttct

SEQ ID NO: 12 - DNA, 354 bp, synthetic construct
  source 1..354: mol_type = other DNA
caggtgcagctggtagagtctgggggcggcttggtgcaggctggggggtctctgagactctcctgtgcagcctctggaatcatcttcagtggcgcgtggatgggctggtaccgccaggctgcaggcgagcagcgcgagttggtcgcatctattactagtggtgatatcacaaactatgcagactccgtgaagggccgattcaccatctctagagacaacgccgaaaacacgggctatctgcaaatgaatacgctgaagcctgaggatacagccgtctattactgtaacgcccgtcctaggggtttaagtttcagttcttactggggccaggggaccctggtcaccgtctcctca

SEQ ID NO: 13 - DNA, 336 bp, synthetic construct
  source 1..336: mol_type = other DNA
ggccccgtgccccctagcaccgccctgcgctacctgatcgaggaactggtgaacatcacccagaaccagaaagcccccctgtgcaacggcagcatggtgtggagcatcaacctgaccgccggcatgtactgtgccgccctggaaagcctgatcaacgtgagcggctgcagcgccatcgagaaaacccagcggatgctgtccggcttctgcccccacaaggtgtccgccggacagttcagcagcctgcacgtgcgggacaccaagatcgaggtggcccagttcgtgaaggacctgctgctgcacctgaagaagctgttccgggagggccggttcaac

SEQ ID NO: 14 - protein, 112 aa, synthetic construct
GPVPPSTALRYLIEELVNITQNQKAPLCNGSMVWSINLTAGMYCAALESLINVSGCSAIEKTQRMLSGFCPHKVSAGQFSSLHVRDTKIEVAQFVKDLLLHLKKLFREGRFN

SEQ ID NO: 15 - protein, 8 aa, synthetic construct
GFTFSSAW

SEQ ID NO: 16 - protein, 116 aa, synthetic construct
QVQLKESGGGLVQAGGSLRLSCVASGFTFSSAWMGWYRQAAGKQRELFASITSSGDTVYAGSVKGRFSISKNNAENTLYLQMDALRPEDTAVYYCNARPGAVNSYWGQGTQVTVST

SEQ ID NO: 17 - protein, 8 aa, synthetic construct
GIIFSGAW

SEQ ID NO: 18 - protein, 8 aa, synthetic construct
ITSSGDTV

SEQ ID NO: 19 - protein, 8 aa, synthetic construct
ITSGGSTV